European Patent Specification EP 3 541 973 B1, published March 27, 2024. Title: POLYNUCLEOTIDE LIBRARIES HAVING CONTROLLED STOICHIOMETRY AND SYNTHESIS THEREOF. Applicant: TWIST BIOSCIENCE CORPORATION. The sequence listing filed with the application follows.

SEQUENCE LISTING (16 sequences)

SEQ ID NO: 1 - DNA, 62 bp, Artificial Sequence
  Description of Artificial Sequence: Synthetic oligonucleotide
  modified_base (51)..(52): Thymidine-succinyl hexamide CED phosphoramidite
agacaatcaaccatttggggtggacagccttgacctctagacttcggcattttttttttttt

SEQ ID NO: 2 - DNA, 112 bp, Artificial Sequence
  Description of Artificial Sequence: Synthetic polynucleotide
  modified_base (101)..(102): Thymidine-succinyl hexamide CED phosphoramidite
cgggatccttatcgtcatcgtcgtacagatcccgacccatttgctgtccaccagtcatgctagccataccatgatgatgatgatgatgagaaccccgcattttttttttttt

SEQ ID NO: 3 - DNA, 19 bp, Artificial Sequence
  Description of Artificial Sequence: Synthetic primer
atgcggggttctcatcatc

SEQ ID NO: 4 - DNA, 20 bp, Artificial Sequence
  Description of Artificial Sequence: Synthetic primer
cgggatccttatcgtcatcg

SEQ ID NO: 5 - DNA, 156 bp, Homo sapiens
cccaccgggactcagattctccccagacgccgaggatggtgctcatggcgccccgaaccctcctcctgctgctctcaggggccctggccctgacccagacctgggcgcgtgagtgcagggtctgcagggaaatgggcgcgtgagtgcagggtctgc

SEQ ID NO: 6 - DNA, 293 bp, Homo sapiens
gctcccaggttcccactccatgaggtatttctacaccaccatgtcccggcccggcgccggggagccccgcttcatctccgtcggctacgtggacgatacgcagttcgtgcggttcgacagcgacgacgcgagtccgagagaggagccgcgggcgccgtggatggagcgggaggggccaaagtattgggaccggaacacacagatctgcaaggcccaggcacagactgaacgagagaacctgcggatcgcgctccgctactacaaccagagcgagggcggtgagttgaccccgg

SEQ ID NO: 7 - DNA, 169 bp, Homo sapiens
tagcagggtcagggttccctcaccttccccccttttcccagccatcttcccagcccaccgtccccatcgtgggcatcgttgctggcttggttctacttgtagctgtggtcactggagctgtggtcgctgctgtaatgtggaggaagaagagctcaggtaaggaaggggt

SEQ ID NO: 8 - DNA, 160 bp, Homo sapiens
gttacccaagaacgcagctgattctccccagacgccgaggatggtgctcatggcgccccgaaccctcctcctgctgctctcaggggccctggccctgacccagacctgggcgcgtgagtgcagggtctgcagggaaatggtagtgtcggaggtcgttcct

SEQ ID NO: 9 - DNA, 160 bp, Homo sapiens
gttacccaagaacgcagctgggttcccactccatgaggtatttctacaccaccatgtcccggcccggcgccggggagccccgcttcatctccgtcggctacgtggacgatacgcagttcgtgcggttcgacagcgacgactagtgtcggaggtcgttcct

SEQ ID NO: 10 - DNA, 160 bp, Homo sapiens
gttacccaagaacgcagctgtggatggagcgggaggggccaaagtattgggaccggaacacacagatctgcaaggcccaggcacagactgaacgagagaacctgcggatcgcgctccgctactacaaccagagcgagggctagtgtcggaggtcgttcct

SEQ ID NO: 11 - DNA, 160 bp, Homo sapiens
gttacccaagaacgcagctgggctacgtggacgatacgcagttcgtgcggttcgacagcgacgacgcgagtccgagagaggagccgcgggcgccgtggatggagcgggaggggccaaagtattgggaccggaacacacagtagtgtcggaggtcgttcct

SEQ ID NO: 12 - DNA, 103 bp, Homo sapiens
gttacccaagaacgcagctgatggcgccccgaaccctcctcctgctgctctcaggggccctggccctgacccagacctgggcgtagtgtcggaggtcgttcct

SEQ ID NO: 13 - DNA, 210 bp, Homo sapiens
aaaaaaaaaaaaaaaaaaaaaaaaagttacccaagaacgcagctgggttcccactccatgaggtatttctacaccaccatgtcccggcccggcgccggggagccccgcttcatctccgtcggctacgtggacgatacgcagttcgtgcggttcgacagcgacgactagtgtcggaggtcgttcctaaaaaaaaaaaaaaaaaaaaaaaaa

SEQ ID NO: 14 - DNA, 210 bp, Homo sapiens
gttacccaagaacgcagctgaaaaaaaaaaaaaaaaaaaaaaaaaggttcccactccatgaggtatttctacaccaccatgtcccggcccggcgccggggagccccgcttcatctccgtcggctacgtggacgatacgcagttcgtgcggttcgacagcgacgacaaaaaaaaaaaaaaaaaaaaaaaaatagtgtcggaggtcgttcct

SEQ ID NO: 15 - DNA, 102 bp, Homo sapiens
gttacccaagaacgcagctgagccatcttcccagcccaccgtccccatcgtgggcatcgttgctggcttggttctacttgtatagtgtcggaggtcgttcct

SEQ ID NO: 16 - DNA, 95 bp, Homo sapiens
gttacccaagaacgcagctggctgtggtcactggagctgtggtcgctgctgtaatgtggaggaagaagagctcagtagtgtcggaggtcgttcct